European Patent Specification EP 3 678 668 B1, published January 10, 2024. Title: ENPP1 Inhibitor Compounds and Methods of Modulating Immune Response. Applicant: The Board of Trustees of the Leland Stanford Junior University Li , Lingyin Smith, Mark Shaw, Kelsey E Carozza, Jacqueline  A Boehnert, Volker. The sequence listing filed with the application follows.

SEQUENCE LISTING (5 sequences)

SEQ ID NO: 1 - DNA, 25 bp, Artificial Sequence
  Synthetic sequence
caccgctggttctatgcacgtctcc

SEQ ID NO: 2 - DNA, 20 bp, Artificial Sequence
  Synthetic sequence
aaactcatgagcagtctgca

SEQ ID NO: 3 - DNA, 22 bp, Artificial Sequence
  Synthetic sequence
aggagatcttcagtttcggagg

SEQ ID NO: 4 - DNA, 20 bp, Artificial Sequence
  Synthetic sequence
gccttccgtgtccccactgc

SEQ ID NO: 5 - DNA, 17 bp, Artificial Sequence
  Synthetic sequence
tgagggggccctcgacg